European Patent Specification EP 3 515 942 B1, published July 30, 2025. Title: Diagnostic anti-PD-L1 antibody and uses thereof. Applicant: Merck Patent GmbH  and Pfizer, Inc. The sequence listing filed with the application follows.

SEQUENCE LISTING (117 sequences)

SEQ ID NO: 1 - protein, 31 aa, Artificial Sequence
  PD-L1 cytoplasmic domain (partial)
RLRKGRMMDVKKCGIQDTNSKKQSDTHLEET

SEQ ID NO: 2 - protein, 15 aa, Artificial Sequence
  PD-L1 cytoplasmic partial cytoplasmic domain
CGIQDTNSKKQSDTH

SEQ ID NO: 3 - protein, 26 aa, Artificial Sequence
  light chain sequence element
AQVLTQTPSPVSASVGSTVTINCQAS

SEQ ID NO: 4 - protein, 8 aa, Artificial Sequence
  light chain sequence element
QSLHRNNY

SEQ ID NO: 5 - protein, 17 aa, Artificial Sequence
  light chain sequence element
LSWFQQKPGQPPKQLIY

SEQ ID NO: 6 - protein, 4 aa, Artificial Sequence
  light chain sequence element with amino acid Xaa being absent
QASX

SEQ ID NO: 7 - protein, 36 aa, Artificial Sequence
  light chain sequence element
TLASGVSSRFSGSGSGTQFTLTISDVVCDDAATYYC

SEQ ID NO: 8 - protein, 10 aa, Artificial Sequence
  light chain sequence element
LGGVSGGPYP

SEQ ID NO: 9 - protein, 24 aa, Artificial Sequence
  heavy chain sequence element
EQLVESGGGLVTPGGSLTLTCTVS

SEQ ID NO: 10 - protein, 8 aa, Artificial Sequence
  heavy chain sequence element
TIDLSTFA

SEQ ID NO: 11 - protein, 17 aa, Artificial Sequence
  heavy chain sequence element
ISWVRQAPGKGLEWIGT

SEQ ID NO: 12 - protein, 7 aa, Artificial Sequence
  heavy chain sequence element
INTDLTT

SEQ ID NO: 13 - protein, 37 aa, Artificial Sequence
  heavy chain sequence element
YYVNWAKGRFTISKTSSTTVDLKMTGLTIEDTATYFC

SEQ ID NO: 14 - protein, 10 aa, Artificial Sequence
  heavy chain sequence element
ARKLFGNGNV

SEQ ID NO: 15 - protein, 236 aa, Artificial Sequence
  light chain sequence
MDTRAPTQLLGLLLLWLPGATVAQVLTQTPSPVSASVGSTVTINCQASQSLHRNNYLSWFQQKPGQPPKQLIYQASTLASGVSSRFSGSGSGTQFTLTISDVVCDDAATYYCLGGVSGGPYPFGGGTEVVVKGDPVAPTVLIFPPAADQVATGTVTIVCVANKYFPDVTVTWEVDGTTQTTGIENSKTPQNSADCTYNLSSTLTLTSTQYNSHKEYTCKVTQGTTSVVQSFNRGDC

SEQ ID NO: 16 - protein, 457 aa, Artificial Sequence
  heavy chain sequence
METGLRWLLLVAVLKGVQCQEQLVESGGGLVTPGGSLTLTCTVSTIDLSTFAISWVRQAPGKGLEWIGTINTDLTTYYVNWAKGRFTISKTSSTTVDLKMTGLTIEDTATYFCARKLFGNGNVWGPGTLVTVSSGQPKAPSVFPLAPCCGDTPSSTVTLGCLVKGYLPEPVTVTWNSGTLTNGVRTFPSVRQSSGLYSLSSVVSVTSSSQPVTCNVAHPATNTKVDKTVAPSTCSKPTCPPPELLGGPSVFIFPPKPKDTLMISRTPEVTCVVVDVSQDDPEVQFTWYINNEQVRTARPPLREQQFNSTIRVVSTLPIAHQDWLRGKEFKCKVHNKALPAPIEKTISKARGQPLEPKVYTMGPPREELSSRSVSLTCMINGFYPSDISVEWEKNGKAEDNYKTTPAVLDSDGSYFLYSKLSVPTSEWQRGDVFTCSVMHEALHNHYTQKSISRSPGK

SEQ ID NO: 17 - DNA, 711 bp, Artificial Sequence
  light chain sequence
atggacacgagggcccccactcagctgctggggctcctgctgctctggctcccaggtgccacagttgcccaagtgctgacccagaccccatcccccgtgtctgcatctgtgggaagcacagtcaccatcaattgccaggccagtcagagtcttcatcgcaacaactacttatcctggtttcagcagaaaccagggcagcctcccaagcaactgatctatcaggcatccactctggcatctggggtctcatcgcggttcagtggcagtggatctgggacacagttcactctcaccatcagcgatgtggtgtgtgacgatgctgccacttactactgtctgggcggtgttagtggtggtccttatcctttcggcggagggaccgaggtggtcgtcaaaggtgatccagttgcacctactgtcctcatcttcccaccagctgctgatcaggtggcaactggaacagtcaccatcgtgtgtgtggcgaataaatactttcccgatgtcaccgtcacctgggaggtggatggcaccacccaaacaactggcatcgagaacagtaaaacaccgcagaattctgcagattgtacctacaacctcagcagcactctgacactgaccagcacacagtacaacagccacaaagagtacacctgcaaggtgacccagggcacgacctcagtcgtccagagcttcaataggggtgactgttag

SEQ ID NO: 18 - DNA, 1374 bp, Artificial Sequence
  heavy chain sequence
atggagactgggctgcgctggcttctcctggtcgctgtgctcaaaggtgtccagtgtcaggagcagctggtggaatccggaggaggcctggtcacgcctgggggatccctgacactcacctgcacagtctctacaatcgacctcagtacctttgcaataagctgggtccgccaggctccagggaaggggctggagtggatcggaaccattaatactgatcttaccacatactatgtgaattgggcgaaaggccgattcaccatctccaaaacctcgtcgaccacggtggatctgaaaatgaccggtctgacaatcgaggacacggccacctatttctgtgccagaaaattatttggaaatggtaatgtctggggcccaggcaccctggtcaccgtctcttcagggcaacctaaggctccatcagtcttcccactggccccctgctgcggggacacacccagctccacggtgaccctgggctgcctggtcaaagggtacctcccggagccagtgaccgtgacctggaactcgggcaccctcaccaatggggtacgcaccttcccgtccgtccggcagtcctcaggcctctactcgctgagcagcgtggtgagcgtgacctcaagcagccagcccgtcacctgcaacgtggcccacccagccaccaacaccaaagtggacaagaccgttgcgccctcgacatgcagcaagcccacgtgcccaccccctgaactcctggggggaccgtctgtcttcatcttccccccaaaacccaaggacaccctcatgatctcacgcacccccgaggtcacatgcgtggtggtggacgtgagccaggatgaccccgaggtgcagttcacatggtacataaacaacgagcaggtgcgcaccgcccggccgccgctacgggagcagcagttcaacagcacgatccgcgtggtcagcaccctccccatcgcgcaccaggactggctgaggggcaaggagttcaagtgcaaagtccacaacaaggcactcccggcccccatcgagaaaaccatctccaaagccagagggcagcccctggagccgaaggtctacaccatgggccctccccgggaggagctgagcagcaggtcggtcagcctgacctgcatgatcaacggcttctacccttccgacatctcggtggagtgggagaagaacgggaaggcagaggacaactacaagaccacgccggccgtgctggacagcgacggctcctacttcctctacagcaagctctcagtgcccacgagtgagtggcagcggggcgacgtcttcacctgctccgtgatgcacgaggccttgcacaaccactacacgcagaagtccatctcccgctctccgggtaaatga

SEQ ID NO: 19 - protein, 8 aa, Artificial Sequence
  epitope
RLRKGRMM

SEQ ID NO: 20 - protein, 8 aa, Artificial Sequence
  epitope
LRKGRMMD

SEQ ID NO: 21 - protein, 8 aa, Artificial Sequence
  epitope
RKGRMMDV

SEQ ID NO: 22 - protein, 8 aa, Artificial Sequence
  epitope
GRMMDVKK

SEQ ID NO: 23 - protein, 8 aa, Artificial Sequence
  epitope
KGRMMDVK

SEQ ID NO: 24 - protein, 8 aa, Artificial Sequence
  epitope
RMMDVKKC

SEQ ID NO: 25 - protein, 8 aa, Artificial Sequence
  epitope
MMDVKKCG

SEQ ID NO: 26 - protein, 8 aa, Artificial Sequence
  epitope
MDVKKCGI

SEQ ID NO: 27 - protein, 8 aa, Artificial Sequence
  epitope
DVKKCGIQ

SEQ ID NO: 28 - protein, 8 aa, Artificial Sequence
  epitope
VKKCGIQD

SEQ ID NO: 29 - protein, 8 aa, Artificial Sequence
  epitope
KKCGIQDT

SEQ ID NO: 30 - protein, 8 aa, Artificial Sequence
  epitope
KCGIQDTN

SEQ ID NO: 31 - protein, 8 aa, Artificial Sequence
  epitope
CGIQDTNS

SEQ ID NO: 32 - protein, 8 aa, Artificial Sequence
  epitope
GIQDTNSK

SEQ ID NO: 33 - protein, 8 aa, Artificial Sequence
  epitope
IQDTNSKK

SEQ ID NO: 34 - protein, 8 aa, Artificial Sequence
  epitope
QDTNSKKQ

SEQ ID NO: 35 - protein, 8 aa, Artificial Sequence
  epitope
DTNSKKQS

SEQ ID NO: 36 - protein, 8 aa, Artificial Sequence
  epitope
TNSKKQSD

SEQ ID NO: 37 - protein, 8 aa, Artificial Sequence
  epitope
NSKKQSDT

SEQ ID NO: 38 - protein, 8 aa, Artificial Sequence
  epitope
SKKQSDTH

SEQ ID NO: 39 - protein, 8 aa, Artificial Sequence
  epitope
KKQSDTHL

SEQ ID NO: 40 - protein, 8 aa, Artificial Sequence
  epitope
KQSDTHLE

SEQ ID NO: 41 - protein, 8 aa, Artificial Sequence
  epitope
QSDTHLEE

SEQ ID NO: 42 - protein, 8 aa, Artificial Sequence
  epitope
SDTHLEET

SEQ ID NO: 43 - protein, 9 aa, Artificial Sequence
  epitope
RLRKGRMMD

SEQ ID NO: 44 - protein, 9 aa, Artificial Sequence
  epitope
LRKGRMMDV

SEQ ID NO: 45 - protein, 9 aa, Artificial Sequence
  epitope
RKGRMMDVK

SEQ ID NO: 46 - protein, 9 aa, Artificial Sequence
  epitope
KGRMMDVKK

SEQ ID NO: 47 - protein, 9 aa, Artificial Sequence
  epiope
GRMMDVKKC

SEQ ID NO: 48 - protein, 9 aa, Artificial Sequence
  epitope
RMMDVKKCG

SEQ ID NO: 49 - protein, 9 aa, Artificial Sequence
  epitope
MMDVKKCGI

SEQ ID NO: 50 - protein, 9 aa, Artificial Sequence
  epitope
MDVKKCGIQ

SEQ ID NO: 51 - protein, 9 aa, Artificial Sequence
  epitope
DVKKCGIQD

SEQ ID NO: 52 - protein, 9 aa, Artificial Sequence
  epitope
VKKCGIQDT

SEQ ID NO: 53 - protein, 9 aa, Artificial Sequence
  epitope
KKCGIQDTN

SEQ ID NO: 54 - protein, 9 aa, Artificial Sequence
  epitope
KCGIQDTNS

SEQ ID NO: 55 - protein, 9 aa, Artificial Sequence
  epitope
CGIQDTNSK

SEQ ID NO: 56 - protein, 9 aa, Artificial Sequence
  epitope
GIQDTNSKK

SEQ ID NO: 57 - protein, 9 aa, Artificial Sequence
  epitope
IQDTNSKKQ

SEQ ID NO: 58 - protein, 9 aa, Artificial Sequence
  epitope
QDTNSKKQS

SEQ ID NO: 59 - protein, 9 aa, Artificial Sequence
  epitope
DTNSKKQSD

SEQ ID NO: 60 - protein, 9 aa, Artificial Sequence
  epitope
TNSKKQSDT

SEQ ID NO: 61 - protein, 9 aa, Artificial Sequence
  epitope
NSKKQSDTH

SEQ ID NO: 62 - protein, 9 aa, Artificial Sequence
  epitope
SKKQSDTHL

SEQ ID NO: 63 - protein, 9 aa, Artificial Sequence
  epitope
KKQSDTHLE

SEQ ID NO: 64 - protein, 9 aa, Artificial Sequence
  epitope
KQSDTHLEE

SEQ ID NO: 65 - protein, 9 aa, Artificial Sequence
  epitope
QSDTHLEET

SEQ ID NO: 66 - protein, 10 aa, Artificial Sequence
  epitope
RLRKGRMMDV

SEQ ID NO: 67 - protein, 10 aa, Artificial Sequence
  epitope
LRKGRMMDVK

SEQ ID NO: 68 - protein, 10 aa, Artificial Sequence
  epitope
RKGRMMDVKK

SEQ ID NO: 69 - protein, 10 aa, Artificial Sequence
  epitope
KGRMMDVKKC

SEQ ID NO: 70 - protein, 10 aa, Artificial Sequence
  epitope
GRMMDVKKCG

SEQ ID NO: 71 - protein, 10 aa, Artificial Sequence
  epitope
RMMDVKKCGI

SEQ ID NO: 72 - protein, 10 aa, Artificial Sequence
  epitope
MMDVKKCGIQ

SEQ ID NO: 73 - protein, 10 aa, Artificial Sequence
  epitope
MDVKKCGIQD

SEQ ID NO: 74 - protein, 10 aa, Artificial Sequence
  epitope
DVKKCGIQDT

SEQ ID NO: 75 - protein, 10 aa, Artificial Sequence
  epitope
VKKCGIQDTN

SEQ ID NO: 76 - protein, 10 aa, Artificial Sequence
  epitope
KKCGIQDTNS

SEQ ID NO: 77 - protein, 10 aa, Artificial Sequence
  epitope
KCGIQDTNSK

SEQ ID NO: 78 - protein, 10 aa, Artificial Sequence
  epitope
CGIQDTNSKK

SEQ ID NO: 79 - protein, 10 aa, Artificial Sequence
  epitope
GIQDTNSKKQ

SEQ ID NO: 80 - protein, 10 aa, Artificial Sequence
  epitope
IQDTNSKKQS

SEQ ID NO: 81 - protein, 10 aa, Artificial Sequence
  epitope
QDTNSKKQSD

SEQ ID NO: 82 - protein, 10 aa, Artificial Sequence
  epitope
DTNSKKQSDT

SEQ ID NO: 83 - protein, 10 aa, Artificial Sequence
  epitope
TNSKKQSDTH

SEQ ID NO: 84 - protein, 10 aa, Artificial Sequence
  epitope
NSKKQSDTHL

SEQ ID NO: 85 - protein, 10 aa, Artificial Sequence
  epitope
SKKQSDTHLE

SEQ ID NO: 86 - protein, 10 aa, Artificial Sequence
  epitope
KKQSDTHLEE

SEQ ID NO: 87 - protein, 10 aa, Artificial Sequence
  epitope
KQSDTHLEET

SEQ ID NO: 88 - protein, 11 aa, Artificial Sequence
  epitope
RLRKGRMMDVK

SEQ ID NO: 89 - protein, 11 aa, Artificial Sequence
  epitope
LRKGRMMDVKK

SEQ ID NO: 90 - protein, 11 aa, Artificial Sequence
  epitope
RKGRMMDVKKC

SEQ ID NO: 91 - protein, 11 aa, Artificial Sequence
  epitope
KGRMMDVKKCG

SEQ ID NO: 92 - protein, 11 aa, Artificial Sequence
  epitope
GRMMDVKKCGI

SEQ ID NO: 93 - protein, 11 aa, Artificial Sequence
  epitope
RMMDVKKCGIQ

SEQ ID NO: 94 - protein, 11 aa, Artificial Sequence
  epitope
MMDVKKCGIQD

SEQ ID NO: 95 - protein, 11 aa, Artificial Sequence
  epitope
MDVKKCGIQDT

SEQ ID NO: 96 - protein, 11 aa, Artificial Sequence
  epitope
DVKKCGIQDTN

SEQ ID NO: 97 - protein, 11 aa, Artificial Sequence
  epitope
VKKCGIQDTNS

SEQ ID NO: 98 - protein, 11 aa, Artificial Sequence
  epitope
KKCGIQDTNSK

SEQ ID NO: 99 - protein, 11 aa, Artificial Sequence
  epitope
KCGIQDTNSKK

SEQ ID NO: 100 - protein, 11 aa, Artificial Sequence
  epitope
CGIQDTNSKKQ

SEQ ID NO: 101 - protein, 11 aa, Artificial Sequence
  epitope
GIQDTNSKKQS

SEQ ID NO: 102 - protein, 11 aa, Artificial Sequence
  epitope
IQDTNSKKQSD

SEQ ID NO: 103 - protein, 11 aa, Artificial Sequence
  epitope
QDTNSKKQSDT

SEQ ID NO: 104 - protein, 11 aa, Artificial Sequence
  epitope
DTNSKKQSDTH

SEQ ID NO: 105 - protein, 11 aa, Artificial Sequence
  epitope
TNSKKQSDTHL

SEQ ID NO: 106 - protein, 11 aa, Artificial Sequence
  epitope
NSKKQSDTHLE

SEQ ID NO: 107 - protein, 11 aa, Artificial Sequence
  epitope
SKKQSDTHLEE

SEQ ID NO: 108 - protein, 11 aa, Artificial Sequence
  epitope
KKQSDTHLEET

SEQ ID NO: 109 - RNA, 23 nt, Artificial Sequence
  IRES
augauaauauggccacaaccaug

SEQ ID NO: 110 - protein, 114 aa, Artificial Sequence
  heavy chain variable region
EQLVESGGGLVTPGGSLTLTCTVSTIDLSTFAISWVRQAPGKGLEWIGTINTDLTTYYVNWAKGRFTISKTSSTTVDLKMTGLTIEDTATYFCARKLFGNGNVWGPGTLVTVSS

SEQ ID NO: 111 - protein, 110 aa, Artificial Sequence
  light chain variable region
AQVLTQTPSPVSASVGSTVTINCQASQSLHRNNYLSWFQQKPGQPPKQLIYQASTLASGVSSRFSGSGSGTQFTLTISDVVCDDAATYYCLGGVSGGPYPFGGGTEVVVK

SEQ ID NO: 112 - protein, 23 aa, Artificial Sequence
  light chain signal sequence
MDTRAPTQLLGLLLLWLPGATVA

SEQ ID NO: 113 - protein, 19 aa, Artificial Sequence
  heavy chain signal sequence
METGLRWLLLVAVLKGVQC

SEQ ID NO: 114 - protein, 213 aa, Artificial Sequence
  MKP1A07310 light chain sequence with signal sequence removed
QVLTQTPSPVSASVGSTVTINCQASQSLHRNNYLSWFQQKPGQPPKQLIYQASTLASGVSSRFSGSGSGTQFTLTISDVVCDDAATYYCLGGVSGGPYPFGGGTEVVVKGDPVAPTVLIFPPAADQVATGTVTIVCVANKYFPDVTVTWEVDGTTQTTGIENSKTPQNSADCTYNLSSTLTLTSTQYNSHKEYTCKVTQGTTSVVQSFNRGDC

SEQ ID NO: 115 - protein, 438 aa, Artificial Sequence
  MKP1A07310 heavy chain sequence with signal peptide removed
QEQLVESGGGLVTPGGSLTLTCTVSTIDLSTFAISWVRQAPGKGLEWIGTINTDLTTYYVNWAKGRFTISKTSSTTVDLKMTGLTIEDTATYFCARKLFGNGNVWGPGTLVTVSSGQPKAPSVFPLAPCCGDTPSSTVTLGCLVKGYLPEPVTVTWNSGTLTNGVRTFPSVRQSSGLYSLSSVVSVTSSSQPVTCNVAHPATNTKVDKTVAPSTCSKPTCPPPELLGGPSVFIFPPKPKDTLMISRTPEVTCVVVDVSQDDPEVQFTWYINNEQVRTARPPLREQQFNSTIRVVSTLPIAHQDWLRGKEFKCKVHNKALPAPIEKTISKARGQPLEPKVYTMGPPREELSSRSVSLTCMINGFYPSDISVEWEKNGKAEDNYKTTPAVLDSDGSYFLYSKLSVPTSEWQRGDVFTCSVMHEALHNHYTQKSISRSPGK

SEQ ID NO: 116 - protein, 10 aa, Artificial Sequence
  MKP1A-7310 Light chain FR4
FGGGTEVVVK

SEQ ID NO: 117 - protein, 11 aa, Artificial Sequence
  MKP1A-7310 heavy chain FR4
WGPGTLVTVSS